European Patent Application EP 4 775 582 A1, published July 15, 2026. Title: 大环化合物及其抗体-药物偶联物. Applicant: 劲方医药科技（上海）有限公司. The sequence listing filed with the application follows.

SEQUENCE LISTING (44 sequences)

SEQ ID NO: 1 - protein, 449 aa, synthetic construct
QVQLQESGPGLVKPSETLSLTCTVSGFSLSNYDVHWVRQAPGKGLEWLGVIWSGGNTDYNTPFTSRLTISVDTSKNQFSLKLSSVTAADTAVYYCARALDYYDYEFAYWGQGTLVTVSSASTKGPSVFPLAPSSKSTSGGTAALGCLVKDYFPEPVTVSWNSGALTSGVHTFPAVLQSSGLYSLSSVVTVPSSSLGTQTYICNVNHKPSNTKVDKRVEPKSCDKTHTCPPCPAPELLGGPSVFLFPPKPKDTLMISRTPEVTCVVVDVSHEDPEVKFNWYVDGVEVHNAKTKPREEQYNSTYRVVSVLTVLHQDWLNGKEYKCKVSNKALPAPIEKTISKAKGQPREPQVYTLPPSREEMTKNQVSLTCLVKGFYPSDIAVEWESNGQPENNYKTTPPVLDSDGSFFLYSKLTVDKSRWQQGNVFSCSVMHEALHNHYTQKSLSLSPGK

SEQ ID NO: 2 - protein, 214 aa, synthetic construct
EIVLTQSPDFQSVTPKEKVTITCRASQSIGTNIHWYQQKPDQSPKLLIKYASESISGIPSRFSGSGSGTDFTLTINSLEAEDAATYYCQQNNEWPTSFGQGTKLEIKRTVAAPSVFIFPPSDEQLKSGTASVVCLLNNFYPREAKVQWKVDNALQSGNSQESVTEQDSKDSTYSLSSTLTLSKADYEKHKVYACEVTHQGLSSPVTKSFNRGEC

SEQ ID NO: 3 - protein, 119 aa, synthetic construct
QVQLQESGPGLVKPSETLSLTCTVSGFSLSNYDVHWVRQAPGKGLEWLGVIWSGGNTDYNTPFTSRLTISVDTSKNQFSLKLSSVTAADTAVYYCARALDYYDYEFAYWGQGTLVTVSS

SEQ ID NO: 4 - protein, 5 aa, synthetic construct
NYDVH

SEQ ID NO: 5 - protein, 16 aa, synthetic construct
VIWSGGNTDYNTPFTS

SEQ ID NO: 6 - protein, 11 aa, synthetic construct
ALDYYDYEFAY

SEQ ID NO: 7 - protein, 110 aa, synthetic construct
EIVLTQSPDFQSVTPKEKVTITCRASQSIGTNIHWYQQKPDQSPKLLIKYASESISGIPSRFSGSGSGTDFTLTINSLEAEDAATYYCQQNNEWPTSFGQGTKLEIKRTV

SEQ ID NO: 8 - protein, 11 aa, synthetic construct
RASQSIGTNIH

SEQ ID NO: 9 - protein, 7 aa, synthetic construct
YASESIS

SEQ ID NO: 10 - protein, 9 aa, synthetic construct
QQNNEWPTS

SEQ ID NO: 11 - protein, 447 aa, synthetic construct
QVQLQQWGAGLLKPSETLSLTCAVYGGSFSGYYWSWIRQPPGKGLEWIGEINHSGSTNYNPSLKSRVTISVETSKNQFSLKLSSVTAADTAVYYCARDKWTWYFDLWGRGTLVTVSSASTKGPSVFPLAPSSKSTSGGTAALGCLVKDYFPEPVTVSWNSGALTSGVHTFPAVLQSSGLYSLSSVVTVPSSSLGTQTYICNVNHKPSNTKVDKRVEPKSCDKTHTCPPCPAPELLGGPSVFLFPPKPKDTLMISRTPEVTCVVVDVSHEDPEVKFNWYVDGVEVHNAKTKPREEQYNSTYRVVSVLTVLHQDWLNGKEYKCKVSNKALPAPIEKTISKAKGQPREPQVYTLPPSREEMTKNQVSLTCLVKGFYPSDIAVEWESNGQPENNYKTTPPVLDSDGSFFLYSKLTVDKSRWQQGNVFSCSVMHEALHNHYTQKSLSLSPGK

SEQ ID NO: 12 - protein, 220 aa, synthetic construct
DIEMTQSPDSLAVSLGERATINCRSSQSVLYSSSNRNYLAWYQQNPGQPPKLLIYWASTRESGVPDRFSGSGSGTDFTLTISSLQAEDVAVYYCQQYYSTPRTFGQGTKVEIKRTVAAPSVFIFPPSDEQLKSGTASVVCLLNNFYPREAKVQWKVDNALQSGNSQESVTEQDSKDSTYSLSSTLTLSKADYEKHKVYACEVTHQGLSSPVTKSFNRGEC

SEQ ID NO: 13 - protein, 117 aa, synthetic construct [sequence omitted]

SEQ ID NO: 14 - protein, 5 aa, synthetic construct
GYYWS

SEQ ID NO: 15 - protein, 16 aa, synthetic construct
EINHSGSTNYNPSLKS

SEQ ID NO: 16 - protein, 9 aa, synthetic construct
DKWTWYFDL

SEQ ID NO: 17 - protein, 116 aa, synthetic construct
DIEMTQSPDSLAVSLGERATINCRSSQSVLYSSSNRNYLAWYQQNPGQPPKLLIYWASTRESGVPDRFSGSGSGTDFTLTISSLQAEDVAVYYCQQYYSTPRTFGQGTKVEIKRTV

SEQ ID NO: 18 - protein, 17 aa, synthetic construct
RSSQSVLYSSSNRNYLA

SEQ ID NO: 19 - protein, 7 aa, synthetic construct
WASTRES

SEQ ID NO: 20 - protein, 9 aa, synthetic construct
QQYYSTPRT

SEQ ID NO: 21 - protein, 702 aa, synthetic construct
QVQLKQSGPGLVQPSQSLSITCTVSGFSLTNYGVHWVRQSPGKGLEWLGVIWSGGNTDYNTPFTSRLSINKDNSKSQVFFKMNSLQSNDTAIYYCARALTYYDYEFAYWGQGTLVTVSSASTKGPSVFPLAPSSKSTSGGTAALGCLVKDYFPEPVTVSWNSGALTSGVHTFPAVLQSSGLYSLSSVVTVPSSSLGTQTYICNVNHKPSNTKVDKRVEPKSCDKTHTCPPCPAPELLGGPSVFLFPPKPKDTLMISRTPEVTCVVVDVSHEDPEVKFNWYVDGVEVHNAKTKPREEQYNSTYRVVSVLTVLHQDWLNGKEYKCKVSNKALPAPIEKTISKAKGQPREPQVYTLPPSRDELTKNQVSLTCLVKGFYPSDIAVEWESNGQPENNYKTTPPVLDSDGSFFLYSKLTVDKSRWQQGNVFSCSVMHEALHNHYTQKSLSLSPGGGGGSGGGGSQVQLQESGGGLVKPGGSLRLSCAASGFTFSSYWMSWVRQAPGKGLEWVANINRDGSASYYVDSVKGRFTISRDDAKNSLYLQMNSLRAEDTAVYYCARDRGVGYFDLWGRGTLVTVSSGGGGSGGGGSGGGGSQSALTQPASVSGSPGQSITISCTGTSSDVGGYNFVSWYQQHPGKAPKLMIYDVSDRPSGVSDRFSGSKSGNTASLIISGLQADDEADYYCSSYGSSSTHVIFGGGTKVTVL

SEQ ID NO: 22 - protein, 214 aa, synthetic construct
DILLTQSPVILSVSPGERVSFSCRASQSIGTNIHWYQQRTNGSPRLLIKYASESISGIPSRFSGSGSGTDFTLSINSVESEDIADYYCQQNNNWPTTFGAGTKLELKRTVAAPSVFIFPPSDEQLKSGTASVVCLLNNFYPREAKVQWKVDNALQSGNSQESVTEQDSKDSTYSLSSTLTLSKADYEKHKVYACEVTHQGLSSPVTKSFNRGEC

SEQ ID NO: 23 - protein, 119 aa, synthetic construct
QVQLKQSGPGLVQPSQSLSITCTVSGFSLTNYGVHWVRQSPGKGLEWLGVIWSGGNTDYNTPFTSRLSINKDNSKSQVFFKMNSLQSNDTAIYYCARALTYYDYEFAYWGQGTLVTVSS

SEQ ID NO: 24 - protein, 5 aa, synthetic construct
NYGVH

SEQ ID NO: 25 - protein, 16 aa, synthetic construct
VIWSGGNTDYNTPFTS

SEQ ID NO: 26 - protein, 11 aa, synthetic construct
ALTYYDYEFAY

SEQ ID NO: 27 - protein, 110 aa, synthetic construct
DILLTQSPVILSVSPGERVSFSCRASQSIGTNIHWYQQRTNGSPRLLIKYASESISGIPSRFSGSGSGTDFTLSINSVESEDIADYYCQQNNNWPTTFGAGTKLELKRTV

SEQ ID NO: 28 - protein, 11 aa, synthetic construct
RASQSIGTNIH

SEQ ID NO: 29 - protein, 7 aa, synthetic construct
YASESIS

SEQ ID NO: 30 - protein, 9 aa, synthetic construct
QQNNNWPTT

SEQ ID NO: 31 - protein, 118 aa, synthetic construct
QVQLQESGGGLVKPGGSLRLSCAASGFTFSSYWMSWVRQAPGKGLEWVANINRDGSASYYVDSVKGRFTISRDDAKNSLYLQMNSLRAEDTAVYYCARDRGVGYFDLWGRGTLVTVSS

SEQ ID NO: 32 - protein, 5 aa, synthetic construct
SYWMS

SEQ ID NO: 33 - protein, 17 aa, synthetic construct
NINRDGSASYYVDSVKG

SEQ ID NO: 34 - protein, 9 aa, synthetic construct
DRGVGYFDL

SEQ ID NO: 35 - protein, 111 aa, synthetic construct
QSALTQPASVSGSPGQSITISCTGTSSDVGGYNFVSWYQQHPGKAPKLMIYDVSDRPSGVSDRFSGSKSGNTASLIISGLQADDEADYYCSSYGSSSTHVIFGGGTKVTVL

SEQ ID NO: 36 - protein, 14 aa, synthetic construct
TGTSSDVGGYNFVS

SEQ ID NO: 37 - protein, 7 aa, synthetic construct
DVSDRPS

SEQ ID NO: 38 - protein, 11 aa, synthetic construct
SSYGSSSTHVI

SEQ ID NO: 39 - protein, 4 aa, synthetic construct
GGFG

SEQ ID NO: 40 - protein, 4 aa, synthetic construct
GGVA

SEQ ID NO: 41 - protein, 4 aa, synthetic construct
KAAN

SEQ ID NO: 42 - protein, 4 aa, synthetic construct
KAAD

SEQ ID NO: 43 - protein, 4 aa, synthetic construct
VKGG

SEQ ID NO: 44 - protein, 5 aa, synthetic construct
GGGGS